European Patent Application EP 4 480 501 A1, published December 25, 2024. Title: Human SIRP alpha nanobodies. Applicant: NMI Naturwissenschaftliches und Medizinisches Institut an. Application EP. The sequence listing filed with the application follows.

SEQUENCE LISTING (43 sequences)

SEQ ID NO: 1 - protein, 8 aa, synthetic construct
EFRLDEYA

SEQ ID NO: 2 - protein, 8 aa, synthetic construct
ISRSGSNT

SEQ ID NO: 3 - protein, 19 aa, synthetic construct
AADLTSHYLSCSSYTDYNS

SEQ ID NO: 4 - protein, 8 aa, synthetic construct
GFSSSYYA

SEQ ID NO: 5 - protein, 8 aa, synthetic construct
ITRSGDTT

SEQ ID NO: 6 - protein, 20 aa, synthetic construct
ALWAWAGSGRLRCTASEYGH

SEQ ID NO: 7 - protein, 8 aa, synthetic construct
GFTLDYYS

SEQ ID NO: 8 - protein, 8 aa, synthetic construct
ITASGSST

SEQ ID NO: 9 - protein, 21 aa, synthetic construct
AAEPCTVVAGILQAPTSDFGS

SEQ ID NO: 10 - protein, 8 aa, synthetic construct
GFTLDYYA

SEQ ID NO: 11 - protein, 9 aa, synthetic construct
ISSDGGGNT

SEQ ID NO: 12 - protein, 21 aa, synthetic construct
AAGPTYYSGSYCRDPHSDYDY

SEQ ID NO: 13 - protein, 8 aa, synthetic construct
GETLDYYA

SEQ ID NO: 14 - protein, 8 aa, synthetic construct
ISSRGDNT

SEQ ID NO: 15 - protein, 21 aa, synthetic construct
VAIKDSWQNYYCSVGWVEYDV

SEQ ID NO: 16 - protein, 8 aa, unidentified
GFTFSSYD

SEQ ID NO: 17 - protein, 8 aa, synthetic construct
IKSGGGRT

SEQ ID NO: 18 - protein, 11 aa, synthetic construct
GSLDNSGAYTG

SEQ ID NO: 19 - protein, 8 aa, synthetic construct
GFSFRDSA

SEQ ID NO: 20 - protein, 7 aa, synthetic construct
IYSDGST

SEQ ID NO: 21 - protein, 12 aa, synthetic construct
APKGVVADEGDY

SEQ ID NO: 22 - protein, 126 aa, synthetic construct
QVQLVESGGGLVQPGGSLRLSCADSEFRLDEYATGWFRQAPGKEREGVACISRSGSNTKYTDSVKGRFTISRDNAKKTVYLQMNSLKPEDTAVYYCAADLTSHYLSCSSYTDYNSWGQGTQVTVSS

SEQ ID NO: 23 - protein, 127 aa, synthetic construct
QVQLVESGGGLVQPGGSLRLSCLVSGFSSSYYAIGWFRQAPGKEREGVSCITRSGDTTNYADSVKGRFTISRDDARNTVYLQMNSLKTEDTAVYSCALWAWAGSGRLRCTASEYGHWGQGTQVTVSS

SEQ ID NO: 24 - protein, 128 aa, synthetic construct
EVQLVESGGGLVQPGGSLRLSCTTSGFTLDYYSVGWFRQAPGKEREGVSCITASGSSTNYANSVKGRFTISRDKVKNTVYLQMSSLKPEDTAVYYCAAEPCTVVAGILQAPTSDFGSWGQGTQVTVSS

SEQ ID NO: 25 - protein, 129 aa, synthetic construct
EVQLVESGGGLVQPGGSLRLSCAASGFTLDYYAIGWFRQVPGKEREGVSCISSDGGGNTYYADSVKGRFTISRDNAKNTVYLQMNSLKPEDSAVYSCAAGPTYYSGSYCRDPHSDYDYWGQGTQVTVSS

SEQ ID NO: 26 - protein, 128 aa, synthetic construct
HVQLVESGGGLVQPGGSLRLSCAASGETLDYYAIGYVRQAPGKEREGVSCISSRGDNTNYADSVKGRFTISRDNANNTVYLQMNSLKPEDTAVYYCVAIKDSWQNYYCSVGWVEYDVWGQGTQVTVSS

SEQ ID NO: 27 - protein, 118 aa, synthetic construct
QVQLQESGGGLVQPGGSLRLACAASGFTFSSYDMSWVRQAPGKGLEWVSDIKSGGGRTYYADSVKGRFTISRDNAKNTVYLQMNSLKPEDTAVYYCGSLDNSGAYTGGGQGSQVTVSS

SEQ ID NO: 28 - protein, 118 aa, synthetic construct
HVQLVESGGGLVQPGGSLRLSCAARGFSFRDSAMSWARQAPGKGLEWVGAIYSDGSTVYEKSVKGRFTISRDNAKNTMYLQMHSLKPEDSARYYCAPKGVVADEGDYSGQGTLVTVSS

SEQ ID NO: 29 - protein, 126 aa, synthetic construct
QVQLVESGGGLVQPGGSLRLSCADSEFRLDEYATGWFRQAPGREREGVACISRSGSNTRYTDSVRGRFTISRDNARRTVYLQMNSLRPEDTAVYYCAADLTSHYLSCSSYTDYNSWGQGTQVTVSS

SEQ ID NO: 30 - protein, 128 aa, synthetic construct
EVQLVESGGGLVQPGGSLRLSCTTSGFTLDYYSVGWFRQAPGREREGVSCITASGSSTNYANSVRGRFTISRDRVRNTVYLQMSSLRPEDTAVYYCAAEPCTVVAGILQAPTSDFGSWGQGTQVTVSS

SEQ ID NO: 31 - protein, 129 aa, synthetic construct
EVQLVESGGGLVQPGGSLRLSCAASGFTLDYYAIGWFRQVPGREREGVSCISSDGGGNTYYADSVRGRFTISRDNARNTVYLQMNSLRPEDSAVYSCAAGPTYYSGSYCRDPHSDYDYWGQGTQVTVSS

SEQ ID NO: 32 - protein, 8 aa, synthetic construct
GRTFRAYA

SEQ ID NO: 33 - protein, 8 aa, synthetic construct
IRWIGGTP

SEQ ID NO: 34 - protein, 20 aa, synthetic construct
AAEETQKGSGLGHDGRHYDY

SEQ ID NO: 35 - protein, 127 aa, synthetic construct
HVQLVESGGGLVQVGDSLRLSCAPSGRTFRAYAMAWFRQAPGKEREFVAAIRWIGGTPSYKDSVKGRFTISRDNARNTFYLQMNSLEPQDTGVYYCAAEETQKGSGLGHDGRHYDYWGQGTPVTVSS

SEQ ID NO: 36 - protein, 34 aa, synthetic construct
YYCAAEETQKGSGLGHDGRHYDYWGQGTPVTVSS

SEQ ID NO: 37 - protein, 33 aa, synthetic construct
YYCAADLTSHYLSCSSYTDYNSWGQGTQVTVSS

SEQ ID NO: 38 - protein, 34 aa, synthetic construct
YSCALWAWAGSGRLRCTASEYGHWGQGTQVTVSS

SEQ ID NO: 39 - protein, 35 aa, unidentified
YYCAAEPCTVVAGILQAPTSDFGSWGQGTQVTVSS

SEQ ID NO: 40 - protein, 35 aa, synthetic construct
YSCAAGPTYYSGSYCRDPHSDYDYWGQGTQVTVSS

SEQ ID NO: 41 - protein, 35 aa, synthetic construct
YYCVAIKDSWQNYYCSVGWVEYDVWGQGTQVTVSS

SEQ ID NO: 42 - protein, 25 aa, synthetic construct
YYCGSLDNSGAYTGGGQGSQVTVSS

SEQ ID NO: 43 - protein, 26 aa, synthetic construct
YYCAPKGVVADEGDYSGQGTLVTVSS